European Patent Specification EP 3 464 333 B1, published May 8, 2024. Title: Seedless fruit producing plants. Applicant: NUNHEMS B. V. The sequence listing filed with the application follows.

SEQUENCE LISTING (22 sequences)

SEQ ID NO: 1 - DNA, 5135 bp, Citrullus lanatus
  exon (1018)..(2088)
  CDS (1018)..(2088)
  Intron (2089)..(2185)
  exon (2186)..(2353)
  CDS (2186)..(2353)
  Intron (2354)..(3098)
  exon (3099)..(3265)
  CDS (3099)..(3265)
  Intron (3266)..(4324)
  exon (4325)..(4607)
  CDS (4325)..(4604)
aaacattcatacttttgaagaaaattagtatattatttatttatattatatttacagattatttattgattattttttaaatatttattgaattttttataatataataaaaatgtcgacatgtcaacacaaaattaatttcatattatgaattagaagtagggaataagagtatgtttggaataaattttcaagtatttaattttaaaaataagtcacttcaaaagaaatataagtgtttggcaaccactcaaactgtattttaaaagccattagtgtctttattataaatacttttcttatcaaaagtgtttaaatgaaaataaaagtttgaagacatttcttttctaggttaatcgaatggcttctaaatttaagatttatcaaatgtatatggtatgtttggttcaaaagagtttttgagcttataattaaagaacatcaatctcatgacttatcaattttttgtaatgtgtatttaaaaaaaaaaagaaataaaaaagaaaaagaaaagaaaaacattttgtaataggaccctacaattaaacaatttaggacatgtctagggagtgattctaaaatagttaaatccacttttgttattattgaaatcacttttaaatatttcaaatcttccaaacacaaaatttattatataaaaattatacttaaaaatgtaaaattaaatactaaattaatttggagtgatttaatatatgttttggggatatatccatttcaaaatcactccaaatatgaatttcataaaattaaagttgaatatttgaaagtagaagactaaaatggaaaagaatatagaggtgaggggccaaaatgatatttaactaaataattattattatttattagattagcacgagaggaggtgacagtgagggaccctctccaaaaaaaaaaaaaactcacttccaattcacaattctcttttgcttcctaacttccataactgctctgctttccatcacgaaactcatcttcatcttcttcattcgaacaatgaagtccaagaagccaagggcaaatcccaaacccgaatcctactctccgccgaagaagaagctccgttctcagcttccacggcgcagacgctctcggatttctccttttttctgctccttggactccgattcccctgctccttctaccaccattgcttttgcttcttcttcctttgctgccgccgaatccagctccacttccttccacgcaggcggacctgaggtttctagccagctcaacgcgtgttttggattccagaggccgaatttgcggaagagacgatttggttcgggtggtgttaatttggatgaagtttcgaagaaggaggttggagtagggagtaatgtggaagtgtctgaatcgtcttgcgttgaatcaaattctggagttgattttggtgttctcggaccaagcactagctccaggttgaagattagaagtgattttaggagaactattgacgaaaatgaagatccaatcgatcaagcggataatggagttgtgaagtttcaattgacggatgctgatgtctcgtcgaagctttgtgaaaagggagctgtgccactcactccttgtggagagtcttgcgctgagtctatcttccagagcgtttgttcgttcgaagagaaaggattagacgttgaagaaaacagactatgggaatttcagttaccagaactaccgagaaatgagatcaatgaaactttcactgtttcgaagtcggattcgacgatagaacagtggcctaatagcttgaagtttgaatcggatcttgcttgcacggagcaattctcttatgagaatgtttcggaatactctagccaggcgttgtccgagcttcaatcaacaattctattggagacgtctgatactgactgctcagattacactccttcaatttttttggaatccggaagcgaattttcagagaaatcgaacgacgacgcagctccttcgtcaacatttagcatgttgctgcagtacagacgcgactttctaaacttaaatgcctctccagacatcagaactagctcgtctattgaagaagagaaagtagatcaatctacggtaattcgctatcttcatgcttccttgacgtttcatttgcaacaaacctgaagctaatcaaacaactatatatatatattatttgattttaaattagattttgagatttgaagaattggacgatgaagaagcctatctaatgttcagaagtagagaaagacgccaattgattattcgcgactacgtagaggagtatcggtccacaacggattatggcgatctcattctccagcaacggtcaaatgtggtccaatggatagttgaagtaagtccttgataccaaaccaccgtgtttctctcaataattcctgaattagcatgagatattttgctccggttttccattttcatcgttaatagcattggtattctgagacattggaactgtttagtgtatcgaggtagtttgaagcactgactctcatatttcaatttgcactgaatcgctaattagttcttaacatctcataaaatgagttcccttgccttatttgctatggaactttatccgacagcgtacttttctgatttggctatcccaacaatgtgatttactaatgaaaattacaaagtcattaccatgatcatactttccactacttaaaagccagcagtttatgatcttgcacctgttacatctagttgttataagctcattctaacgaatgaggcctgccaccagcacaacgcatctggcatcttgaatcaactaagtttaactgatttttcatttcttttcttacttctgcttgaatatattttctgtttgtttttcatcttaataatagaatacagattcataaccgcgagatttgtgcttattactgtggatgttgacattttcttaggaatactccaatgtagttgcattttcatcatctgttgacgtttctagttcaaggaatacattctttatactatttttattccttttctgcgttaatacttgtcaccaaccaattgggtcaaattttttacattatgttgctttgttttgttgaatgatgcagcgatcgagagattccaaacttcatcaggagacgacatttttaggagttaccctcctggaccagattctgagcagaggattcttcaaagctggaagacaccttcaaattctgggcatagcatgtctaactttggcgactagaattgaagaaaatcagtcatacagctggtgactttttttctatcttttgtctatttgtgtgcatctcagttttaactatataacaagtgttgttcttatctactgtaacttcaacttaacttcgttagtatgatgaatattgcttgaaaacaaactgtatgccagttggtcttcttgtttcgatccaagggagtgaaattgggtaagttaggatcgaatgctaagtagtactagaaataataatcagaaagaattgtattaaagtaattgaatctaatagtcttgaatattttttctaaagttcaaagtgtcgagcctgaaagctttgcgtttacatggaccaaagtaatgttgtgaatatatcgtaggtcctcttatagcaattatgtaacaaataatagccatacattagtgtcgatacacaccacccgtacggtactgtagtcgaatattgccataacactatctttcagttcttatgttaacaattcatgtgcacagaagagacccgagacccaccaagaaaacattatctttgacttgtatatagaactctaagtcgagtcaaatgtaaaacaattctttttcttctcttctctttctcaaacttccttttgtagccttcatttatctttgacttgcaatttacatgcaaaatgttaaataattgtgatttgtttaattaaatagagccttgtgaattgagaaggtatccaagctagctggtgggtctcgagcttggtggatatatttataaagctatgataggactgatttgttttatttttgggcatttcagggtgcagcaaaggaatatccgtgtagagagcaacacgtacagaagatctgaagttgttggcatggaatggcttgttgaagaagtcttaaagttccattgtttcttgccaactgtttacaacttcttatggtacatcttcctttgactaacttgaccattggtgggaagggaaaaagttttccctttcgtgcatccattttcaataaactccttccgcccattaacaatttgaatctactgcgaataacatgctttatttaattttctttttttgaaaattatcttaggttctacctgaaagctgctggagctgactcgaatttggagaatcgagctaagaactttgcggagctggttctttcagacaaagtccaattttgttatttcccttcaactattgcagctgcggttgtcatcttggcgtccctaggagaaaaacaagatgcaccaagtcaacgagtcattgaggtacataaatacaaatacctgttagagagaaaactcctttatctttatattgacccaattgaacaaataaacaagtattttgaaatcgagaagaaactttaaagttttacaaaaacaccataatctaaatccaattagattcaactgtaatgtaaagtacaataataaaatacatataccataaggaaatggtaggttatagtgtttgtttcaattagatattcaatttatatattagttagtgttgttaatctccctgaatatttcttactaacttgaggaaggtctcctgtcttctggaaacccttccatgcccaaaatttcagccttctgctattcccattaagtcaaacatgtaatgagtttacttttctttctccttctaattattaattatttttaataatttatttgtctaattcattttctgtagtctgaacccacgaacttgcttatcacaaaatccaaaaccaaaaaccccatcacaattttggaaatctttttgagaactgctactataaccatgtaatttctttcaaaatctacaaaaatagaaataacacttatttagactatctgtggtactatctcataacatctggtgcattgtggctttgcagacgcatgtca

SEQ ID NO: 2 - protein, 562 aa, Citrullus lanatus
MKSKKPRANPKPESYSPPKKKLRSQLPRRRRSRISPFFCSLDSDSPAPSTTIAFASSSFAAAESSSTSFHAGGPEVSSQLNACFGFQRPNLRKRRFGSGGVNLDEVSKKEVGVGSNVEVSESSCVESNSGVDFGVLGPSTSSRLKIRSDFRRTIDENEDPIDQADNGVVKFQLTDADVSSKLCEKGAVPLTPCGESCAESIFQSVCSFEEKGLDVEENRLWEFQLPELPRNEINETFTVSKSDSTIEQWPNSLKFESDLACTEQFSYENVSEYSSQALSELQSTILLETSDTDCSDYTPSIFLESGSEFSEKSNDDAAPSSTFSMLLQYRRDFLNLNASPDIRTSSSIEEEKVDQSTILRFEELDDEEAYLMFRSRERRQLIIRDYVEEYRSTTDYGDLILQQRSNVVQWIVERSRDSKLHQETTFLGVTLLDQILSRGFFKAGRHLQILGIACLTLATRIEENQSYSWFYLKAAGADSNLENRAKNFAELVLSDKVQFCYFPSTIAAAVVILASLGEKQDAPSQRVIEVHKYKYLLERKLLYLYIDPIEQINKYFEIEKKL

SEQ ID NO: 3 - RNA, 1673 nt, Artificial Sequence
  Induced by mutation
  mRNA (1)..(1673)
  CDS (1)..(1098)
augaaguccaagaagccaagggcaaaucccaaacccgaauccuacucuccgccgaagaagaagcuccguucucagcuuccacggcgcagacgcucucggauuucuccuuuuuucugcuccuuggacuccgauuccccugcuccuucuaccaccauugcuuuugcuucuucuuccuuugcugccgccgaauccagcuccacuuccuuccacgcaggcggaccugagguuucuagccagcucaacgcguguuuuggauuccagaggccgaauuugcggaagagacgauuugguucgggugguguuaauuuggaugaaguuucgaagaaggagguuggaguagggaguaauguggaagugucugaaucgucuugcguugaaucaaauucuggaguugauuuugguguucucggaccaagcacuagcuccagguugaagauuagaagugauuuuaggagaacuauugacgaaaaugaagauccaaucgaucaagcggauaauggaguugugaaguuucaauugacggaugcugaugucucgucgaagcuuugugaaaagggagcugugccacucacuccuuguggagagucuugcgcugagucuaucuuccagagcguuuguucguucgaagagaaaggauuagacguugaagaaaacagacuaugggaauuucaguuaccagaacuaccgagaaaugagaucaaugaaacuuucacuguuucgaagucggauucgacgauagaacaguggccuaauagcuugaaguuugaaucggaucuugcuugcacggagcaauucucuuaugagaauguuucggaauacucuagccaggcguuguccgagcuucaaucaacaauucuauuggagacgucugauacugacugcucagauuacacuccuucaauuuuuuuggaauccggaagcgaauuuucagagaaaucgaacgacgacgcagcuccuucgucaacauuuagcauguugcugcaguacagacgcgacuuucuaaacuuaaaugccucuccagacaucagaacuagcucgucuauugaagaagagaaaguagaucaaucuacgaauuggacgaugaagaagccuaucuaauguucagaaguagagaaagacgccaauugauuauucgcgacuacguagaggaguaucgguccacaacggauuauggcgaucucauucuccagcaacggucaaaugugguccaauggauaguugaacgaucgagagauuccaaacuucaucaggagacgacauuuuuaggaguuacccuccuggaccagauucugagcagaggauucuucaaagcuggaagacaccuucaaauucugggcauagcaugucuaacuuuggcgacuagaauugaagaaaaucagucauacagcugguucuaccugaaagcugcuggagcugacucgaauuuggagaaucgagcuaagaacuuugcggagcugguucuuucagacaaaguccaauuuuguuauuucccuucaacuauugcagcugcgguugucaucuuggcgucccuaggagaaaaacaagaugcaccaagucaacgagucauugagguacauaaauacaaauaccuguuagagagaaaacuccuuuaucuuuauauugacccaauugaacaaauaaacaaguauuuugaaaucgagaagaaacuuuaa

SEQ ID NO: 4 - protein, 365 aa, Artificial Sequence
  Synthetic Construct
MKSKKPRANPKPESYSPPKKKLRSQLPRRRRSRISPFFCSLDSDSPAPSTTIAFASSSFAAAESSSTSFHAGGPEVSSQLNACFGFQRPNLRKRRFGSGGVNLDEVSKKEVGVGSNVEVSESSCVESNSGVDFGVLGPSTSSRLKIRSDFRRTIDENEDPIDQADNGVVKFQLTDADVSSKLCEKGAVPLTPCGESCAESIFQSVCSFEEKGLDVEENRLWEFQLPELPRNEINETFTVSKSDSTIEQWPNSLKFESDLACTEQFSYENVSEYSSQALSELQSTILLETSDTDCSDYTPSIFLESGSEFSEKSNDDAAPSSTFSMLLQYRRDFLNLNASPDIRTSSSIEEEKVDQSTNWTMKKPI

SEQ ID NO: 5 - DNA, 2348 bp, Cucumis melo
  CDS (192)..(1925)
  ref <308>: GenBank/XM_008454203.1
  ref <309>: 2014-06-25
  ref <313>: (1)..(2348)
aactgataaaaacattccaaattgagggatcaaaatgatattttacacgaaaaggaggaggagggtgggacccacttcgagagaaacctcaattcgaattcacatttctcccttcgcttctttaacttcctaactgctctgctttccatcacgaaactccatcttcatcttcctccttaatcgcaaacaccatgaaatccaagaaacgaaggcctaatcccaaccctcaatccttctctccacccaagaacaagaagctccgttctcaccttccacgccgcaaacgcccgaggatttcaccttttctctgctctaatttggtttcccattcccccgctccctccaccacctttgctttggctgccgcagaatccacctccacttccttctacacatcccgacctgacgtttctagccacctcagcgctcccaatttcaggaagagacgatttgattccaagaaggaggttggagtagggagtaatgtggaagtgtctgaatcttcttgtgttgaatctaattctggagttgattttggtgtttccggaccaagcactacttcgaagttaaagaataggagtagttttaggacaactattaacggaaatgaagatcaaattgatccagcggagaatggagttgagaagttcgaattcacggatgttgatgtctcgtcgaagctttgtggaaaggaagctgtggtactcacttcttgtgtagagtcttgtgctgaatctatctttcagagtgtttgtccgttcgaagagaaacgattagaagttgaagataacagactatgggaatttcagttacctgagctaccgagaaatgagattaatgaaactttcactgtttcgaagtcggattcgacgatagaacagtggcctggcagcttgaagtttgaatcggatcttgcttgcacggagcaattctcttacgatgatgtttcggaatactctagccaggcgttgtcgcttcagtcaactattctattggagacttctgatgagtactgctcagattacactccatcaattttcttggaatccggaagcgaattttcagagaaatcgaacgaagacgcagctccttcatcgacatttagaatgttgctgcagtacagacgcgactttctaagcttaaattcctctccagacatcagaactagctcgcctattgaagaagaaaaagtagatcaatctacgattctgagatttgaagaattggacgacgaagaagcctatcgaatgttcagaaatagagaaagacgccaattgattattcacgactacatagaggagtatcgatccacaacggattatggcgatctcattcttcagcaacggtcaaatatggtccaatggatagttgaacgatctagagaaaacaaacttcatcaggagacgacatttttaggagttacccttctagaccagattctgagcaaaggattcttcaaagctgaaagtcgccttcaaattctaggcatagcatgtctaactttggcgactagaattgaagaaaatcagtcatacagctggttacagcaaaggaatatccatgtagggagcaacacgtacagaagagcagaagttgttggcatggaatggcttgttgaagaagttcttaagttccattgtttcttgccaactgtttacaacttcttgtggttctacctgaaagctgctggagctaactcagatttggagaatcgagctaagaatttcgcagtgctcgttcttgcagacaaagtccaattttgttatttcccttcaacaattgcagctgcagttgtcatcttggcgtccttaggagaaaaacaagatgcaccaagtcaacgagtcattgagacacatgtcagaacagaaaacgacgatctgcctgaatgtatcgagagcttggagtggctattaaagcttttatgatggaagcatcaaatcctaacacagcaaaaaagaaagcaagcaattggtctttttgacatattcttgaccacttaaacatcatcttgaacacagctagtgaagctcaccctccgaaaccagctatataggtaagacattcatcaattcagttctcttctattctatcaccaacagaatgaaaatttggtttttcctttcaaattttattataacaagagattgaatcaggacctagtcaagtccaaaaccaaatagtatttgatgttcatttacatgctttcataatttcatgtatttagtagtgttgaattacaggatgtatgtaattgatactcagacctaatgactctatattcttcaccaaaacaaacaatggttacgatgagattttcaatactcgagcaattgaagcttaaaatgtaa

SEQ ID NO: 6 - protein, 577 aa, Cucumis melo
MKSKKRRPNPNPQSFSPPKNKKLRSHLPRRKRPRISPFLCSNLVSHSPAPSTTFALAAAESTSTSFYTSRPDVSSHLSAPNFRKRRFDSKKEVGVGSNVEVSESSCVESNSGVDFGVSGPSTTSKLKNRSSFRTTINGNEDQIDPAENGVEKFEFTDVDVSSKLCGKEAVVLTSCVESCAESIFQSVCPFEEKRLEVEDNRLWEFQLPELPRNEINETFTVSKSDSTIEQWPGSLKFESDLACTEQFSYDDVSEYSSQALSLQSTILLETSDEYCSDYTPSIFLESGSEFSEKSNEDAAPSSTFRMLLQYRRDFLSLNSSPDIRTSSPIEEEKVDQSTILRFEELDDEEAYRMFRNRERRQLIIHDYIEEYRSTTDYGDLILQQRSNMVQWIVERSRENKLHQETTFLGVTLLDQILSKGFFKAESRLQILGIACLTLATRIEENQSYSWLQQRNIHVGSNTYRRAEVVGMEWLVEEVLKFHCFLPTVYNFLWFYLKAAGANSDLENRAKNFAVLVLADKVQFCYFPSTIAAAVVILASLGEKQDAPSQRVIETHVRTENDDLPECIESLEWLLKLL

SEQ ID NO: 7 - DNA, 38 bp, Artificial Sequence
  Primer
gtaaaacgacggccagttgcctctccagacatcagaac

SEQ ID NO: 8 - DNA, 38 bp, Artificial Sequence
  Primer
caggaaacagctatgaccaatccgttgtggaccgatac

SEQ ID NO: 9 - DNA, 38 bp, Artificial Sequence
  Primer
gtaaaacgacggccagtgctccttcgtcaacatttagc

SEQ ID NO: 10 - DNA, 40 bp, Artificial Sequence
  Primer
caggaaacagctatgaccttggcgtctttctctacttctg

SEQ ID NO: 11 - DNA, 38 bp, Artificial Sequence
  Primer
caggaaacagctatgaccctggtccaggagggtaactc

SEQ ID NO: 12 - protein, 569 aa, Cucumis sativus
MKSKKRRPNPKPQSFSPPKNKKLRSQLPRRKRPLILPFFCCYLDSDSPPPSTTFSFASSSSFTAAQSTSTSFFPTGPEVSSHLNPLNFRKTRFDSNKEVGVGSNEQVSESSCVESNSGLDFGVSGPSTTSKLKNRRTIHGNEDPIDPAENGVDASSKLCGKGAVVLTSCVESCAESIFQSVCSFEEKGLEVEDNRLWEFQLPELQKNEINKTFTVSKSDSTIEQWPGSLKIESDLACTEQFSYDDVSEYLSQPLSLQSTILLEMSDDCSDYTPSIFLESGSEFSEKSNEDAAPTSTFTMLLQYRREFISLNFSHIRTSSSIEEEEVDQSTILRFEELDDEEAYRMFRNRERRQLIICDYIEEYRSTTDYGDFILQQRSNMVQWIVERSREKKLHQETTFLGVTLLDQILSKGFFKAETHLQILGIACLTLATRIEENQSYSWLQQRNIHVGSNTYRRSKVVGMEWLVEEVLKFHCFLPTVYNFLWFYLKAAGANSDLENRAKNFAVLVLAEKVQFCYFPSTIAAAVVILASLGEKQDAPSERVIEIHVRTENDDLPECIESLEWLLKFL

SEQ ID NO: 13 - DNA, 50 bp, artificial
  sequence of sample 114 and 115 of Figure 2
acgattttgagatttgaagaattggacgatgaagaagcctatctaatgtt

SEQ ID NO: 14 - protein, 17 aa, artificial
  sequence of sample 114 and 115 of Figure 2
TILRFEELDDEEAYLMF

SEQ ID NO: 15 - DNA, 34 bp, artificial
  sequence of sample 116 and 117 of Figure 2
acgaattggacgatgaagaagcctatctaatgtt

SEQ ID NO: 16 - protein, 9 aa, artificial
  sequence of sample 116 and 117 of Figure 2
TNWTMKKPI

SEQ ID NO: 17 - DNA, 1689 bp, artificial
  Citrullus lanatus - cDNA of cyclin SDS like gene comprising a C to T mutation of  nucleotide 670 resulting in a STOP codon
  CDS (1)..(672)
atgaagtccaagaagccaagggcaaatcccaaacccgaatcctactctccgccgaagaagaagctccgttctcagcttccacggcgcagacgctctcggatttctccttttttctgctccttggactccgattcccctgctccttctaccaccattgcttttgcttcttcttcctttgctgccgccgaatccagctccacttccttccacgcaggcggacctgaggtttctagccagctcaacgcgtgttttggattccagaggccgaatttgcggaagagacgatttggttcgggtggtgttaatttggatgaagtttcgaagaaggaggttggagtagggagtaatgtggaagtgtctgaatcgtcttgcgttgaatcaaattctggagttgattttggtgttctcggaccaagcactagctccaggttgaagattagaagtgattttaggagaactattgacgaaaatgaagatccaatcgatcaagcggataatggagttgtgaagtttcaattgacggatgctgatgtctcgtcgaagctttgtgaaaagggagctgtgccactcactccttgtggagagtcttgcgctgagtctatcttccagagcgtttgttcgttcgaagagaaaggattagacgttgaagaaaacagactatgggaattttagttaccagaactaccgagaaatgagatcaatgaaactttcactgtttcgaagtcggattcgacgatagaacagtggcctaatagcttgaagtttgaatcggatcttgcttgcacggagcaattctcttatgagaatgtttcggaatactctagccaggcgttgtccgagcttcaatcaacaattctattggagacgtctgatactgactgctcagattacactccttcaatttttttggaatccggaagcgaattttcagagaaatcgaacgacgacgcagctccttcgtcaacatttagcatgttgctgcagtacagacgcgactttctaaacttaaatgcctctccagacatcagaactagctcgtctattgaagaagagaaagtagatcaatctacgattttgagatttgaagaattggacgatgaagaagcctatctaatgttcagaagtagagaaagacgccaattgattattcgcgactacgtagaggagtatcggtccacaacggattatggcgatctcattctccagcaacggtcaaatgtggtccaatggatagttgaacgatcgagagattccaaacttcatcaggagacgacatttttaggagttaccctcctggaccagattctgagcagaggattcttcaaagctggaagacaccttcaaattctgggcatagcatgtctaactttggcgactagaattgaagaaaatcagtcatacagctggttctacctgaaagctgctggagctgactcgaatttggagaatcgagctaagaactttgcggagctggttctttcagacaaagtccaattttgttatttcccttcaactattgcagctgcggttgtcatcttggcgtccctaggagaaaaacaagatgcaccaagtcaacgagtcattgaggtacataaatacaaatacctgttagagagaaaactcctttatctttatattgacccaattgaacaaataaacaagtattttgaaatcgagaagaaactttaa

SEQ ID NO: 18 - protein, 223 aa, artificial
  Synthetic Construct
MKSKKPRANPKPESYSPPKKKLRSQLPRRRRSRISPFFCSLDSDSPAPSTTIAFASSSFAAAESSSTSFHAGGPEVSSQLNACFGFQRPNLRKRRFGSGGVNLDEVSKKEVGVGSNVEVSESSCVESNSGVDFGVLGPSTSSRLKIRSDFRRTIDENEDPIDQADNGVVKFQLTDADVSSKLCEKGAVPLTPCGESCAESIFQSVCSFEEKGLDVEENRLWEF

SEQ ID NO: 19 - protein, 590 aa, artificial
  Solanum lycopersicum
MKRKLHAEAVQPAVQQPKEILPAVKRQLRSKLPRRKRSHISPILRSFSIAASSYLTSEVSRQSSKGSVNKEVKKREIEGEEFRRITRAYFRKKLLVDQKKDSEVELSECSCVDSCSEVIGKIIKIEDPVDISRDIVSKRNRNAKVIEGTEDSEVISRFLKASGGFCGESSKSGEDAVARSRNAAKIIHEDVVSFNSVLQSPSESKCGNLSVQSIKCSENRAAEEVESEVSRVCPEVELSAVEQAHEKLVEAELDLECSENFSIVDVSDDYSSAYSELQSEIFPESSDIDISDYSPSYWYDSGSQFSEKSNADASPSPTFTLFLRFGQQFCRSTAALQSTPINSSEDQISTEFTGLEDEEDEESYRMIRNRERRQLYLHDYAEEYCSTTDYGDLIVQQRLQMVHWILEQATRKDLQKETMFLSVNLFDRFLSKGYFKTKRCLQIAGIACLTLAVRIEENQPFNSIRQKTFSVAGTTYSCSEVVAMEWLVQEVLNFQCFLPTIYNFLWFYLKAATATEYMEKTAKYLAVLALLGHEHLCYRPSTVASALVILALSAANLYASCHLVTKTHAKIEDEDLPECIKSLEWLVKYI

SEQ ID NO: 20 - protein, 560 aa, Capsicum annuum
MKRNLHAEAAEILPAMKKQLRSKLPRRKRSHISPILLSVNKETVVVVKKKREIEVDEFRRITRAYLKKKDAEVELSECSCVDSCSEIVGKIVKIEDPVDISHDIVSKQKRNAKVVEGTEDSDAISFLKNASGFFGESSKSGVDVSVEGSRTTEKINDEDVVSFNSVLQSPSESKCGNLSVQTIKCTENRAAEEDIESEVSRIYPEVELSALENANEKLVEPEFDLECSENFSVLDVTADYSSAYSELQSEIFPESSDFDLSDYSPSYWYDSGSQFSEKSNGDATPSPTLTLFLRFSQQFCRSTAALQFTSVNSSEDHISTEITGLKDEEDEESYMLIRNRERRQLYLHDYAEEYCSTTDSGDLIVQQRLLMVHWILEQATRKDLLKETMFLSVNLFDRFLSKGYFKTKRCLQIVGIACLTLAVRIEENQPFNSIRQKTFTVAGTAYSCSEVVAMEWLVQEVLNFQCFLPTIYNFLWFYLKAARATEYMERTTKYLAVLALLGHEHLCYRPSTVASALVILALSAANLYVSCHLVTKTHAKIKDEDLPECIKSLEWLVKYI

SEQ ID NO: 21 - DNA, 23 bp, artificial
  Forward primer
cgaagagaaaggattagacgttg

SEQ ID NO: 22 - DNA, 22 bp, artificial
  reverse primer
tctgagcagtcagtatcagacg